European Patent Specification EP 3 609 909 B1, published July 2, 2025. Title: LACTASE ENZYMES WITH IMPROVED PROPERTIES. Applicant: Chr. Hansen A/S. The sequence listing filed with the application follows.

SEQUENCE LISTING (41 sequences)

SEQ ID NO: 1 - protein, 1049 aa, Bifidobacterium adolescentis
MADTAELAIVHATTASASWLTDPTVFAANRKPAHSSHRYVIGETSEPKQSLDGEWKVRIEQARNVDVESAPFAAVDFEDGDFGAIEVPGHLQMAGYLKNKYVNIQYPWDGHEDPQAPNIPENNHVAIYRRRFALDAQLARTLENDGTVSLTFHGAATAIYVWLDGTFVGYGEDGFTPSEFDVTEALRNGNGNAADSPEAEHTLTVACYEYSSASWLEDQDFWRLHGLFRTVELAAQPHTHVETVQLEADYTAADTAGTADTAELNAALTLRNSADAMTIESTLRDGDGNVVWESTQACNGEIALNSGKMTNIAPWSAESPTLYTLTVRVVGHDGAIIETVTQKIGFRTFRIENGIMTLNGKRIVFKGADRHEFDAKRGRAITREDMLSDVVFCKRHNINAIRTSHYPNQEYWYDLCDEYGLYLIDETNMETHGTWVANNVERPEDGIPGSRPEWEGACVDRINSMMRRDYNHPSVLIWSLGNESSAGEVFRAMYRHAHTIDPNRPVHYEGSVHMREFEDVTDIESRMYAHADEIERYLNDGSPAHTDGPKKPYISCEYMHAMGNSCGNMDEYTALERYPMYQGGFIWDFIDQAIETKLPDGTTRMCYGGDFGDRPSDYEFSGDGLLFADRTPSPKAQEVKQLYANVKIVVSVDEARITNDNLFVSTGDYRFVLRILADGKPVWSTTRRFDVAAGESASFEVDWPVDDYRSNAEELVLEVSQQLGNACDWAPAGYELAFGQCVVAGAKTTADAVDAAGAPADGTVTLGRWNAGVRGQGREALFSRTQGGMVSYTFGEREFVLRRPSITTFRPLTDNDRGAGHAFERAAWAVAGKYARCVDCAIANRGENAVEATYTYELAIPQRTKVTVRYVADTAGLVSLDVEYPGEKNGDLPTIPAFGIEWALPVEYANLRFYGAGPEETYADRRHAKLGVWSTTAGDDCAPYLLPQETGNHEDVRWAEITDDSGHGVRVKRGAGAKPFAMSLLPYSSTMLEEALHQDELPKPRHMFLRLLAAQMGVGGDDSWMSPVHEQYQLPADQPLSLNVQLKLF

SEQ ID NO: 2 - protein, 625 aa, Lactobacillus sakei
MQPNIQWLDTPAVFRVGQLPAHSDHRYYATLAEMAQQQSSFEQSLNGTWQFHYSVNAASRPKSFYELAFDAQDFEPITVPQHIELAGYEQLHYINTMYPWEGHYYRRPAFSTSDDKQHLGMFSEADYNPVGSYLHHFDLTPALRNQRVIIRFEGVEQAMYVWLNGQFIGYAEDSFTPSEFDLTPYLKETDNCLAVEVHKRSSAAFIEDQDFFRFFGIFRDVKLLAKPRTHLEDLWVIPEYDVVQQTGQVKLRLQFSGDENRVHLRIRDQHQIILTADLTSAAQVNGLYKMPELVQAWSNQTPNLYTLELEVVDQAGETIEISQQPFGFRKIEIKDKVMLLNGKRLVINGVNRHEWHPETGRTITAEDEAWDIACMQRNHINAVRTSHYPDRLSFYNGCDQAGIYMMAETNLESHGSWQKMGAVEPSWNVPGSYDEWEAATLDRARTNFETFKNHVSILFWSLGNESYAGSVLEKMNAYYKQQDPTRLVHYEGVFRAPEYKATISDVESRMYATPAEIKAYLDNAPQKPFILCEYMHDMGNSLGGMQSYIDLLSQYDMYQGGFIWDFIDQALLVTDPVTGQRELRYGGDFDDRPSDYEFSGDGLVFATRDEKPAMQEVRYYYGEHK

SEQ ID NO: 3 - protein, 330 aa, Lactobacillus sakei
MKNQQCRRLDTIMANTNKRLAVIFGDVTLGLKGPDFHYLFSYQTGGPESLRIQGKEWLYRSPKPTFWRATTDNDRGNQFPLKSGMWLAADQFIACQSITVAIDGQTIPLPIAPENNRYSGQETAQEVTVTYTYQTITTPQTTVEVSYTIQASGKIRVAVTYHGQAGLPSLPVFGLRFVMPTPATRFIYQGLSGETYPDRMAGGMAGEYEVTGLPVTPYLVPQDCGVHMATDWVTIYRQAVLDNRLREPVETGLKFKMVDQPFAFSCLPYTAEELENATHHSELPAPHRTVLSLLGAVRGVGGIDSWGSDVEAAYQIDATQDHHLEFEISF

SEQ ID NO: 4 - protein, 1049 aa, Bifidobacterium adolescentis
MADTAELAIVHATTASASWLTDPTVFAANRKPAHSSHRYVIGETSEPKQSLDGEWKVRIEQARNVDVESAPFAAVDFEDGDFGAIEVPGHLQMAGYLKNKYVNIQYPWDGHEDPQAPNIPENNHVAIYRRRFALDAQLARTLENDGTVSLTFHGAATAIYVWLDGTFVGYGEDGFTPSEFDVTEALRNGNGNAADSPEAEHTLTVACYEYSSASWLEDQDFWRLHGLFRTVELAAQPHTHVETVQLEADYTAADTAGTADTAELNAALTLRNPADAMTIESTLRDGDGNVVWESTQACNGEIALNSGKMTNIAPWSAESPTLYTLTVRVVGHDGAIIETVTQKIGFRTFRIENGIMTLNGKRIVFKGADRHEFDAKRGRAITREDMLSDVVFCKRHNINAIRTSHYPNQEYWYDLCDEYGLYLIDETNMETHGTWVANNVERPEDGIPGSRPEWEGACVDRINSMMRRDYNHPSVLIWSLGNESSAGEVFRAMYRHAHTIDPNRPVHYEGSVHMREFEDVTDIESRMYAHADEIERYLNDGSPAHTDGPKKPYISCEYMHAMGNSCGNMDEYTALERYPMYQGGFIWDFIDQAIETKLPDGTTRMCYGGDFGDRPSDYEFSGDGLLFADRTPSPKAQEVKQLYANVKIAVSVDEARITNDNLFVSTGDYRFVLRILADGKPVWSTTRRFDVAAGESASFEVDWPVDDYRSNAEELVLEVSQQLGNACDWAPAGYELAFGQCVVAGAKTTADAVDAAGAPADGTVTLGRWNAGVRGQGREALFSRTQGGMVSYTFGEREFVLRRPSITTFRPLTDNDRGAGHAFERAAWAVAGKYARCVDCAIANRGENAVEATYTYELAIPQRTKVTVRYVADTAGLVSLDVEYPGEKNGDLPTIPAFGIEWALPVEYANLRFYGAGPEETYADRRHAKLGVWSTTAGDDCAPYLLPQETGNHEDVRWAEITDDSGHGVRVKRGAGAKPFAMSLLPYSSTMLEEALHQDELPKPRHMFLRLLAAQMGVGGDDSWMSPVHEQYQLPADQPLSLNVQLKLF

SEQ ID NO: 5 - protein, 626 aa, Lactobacillus amylovorus
MKANIKWLDDPEVFRINQLPAHSDHPFYKDYREWQNHSSSFKQSLNGAWQFHFSKDPQSRPIDFYKRSFDSSSFDTIPVPSEIELNGYAQNQYTNILYPWESKIYRKPAYTLGRGIKDGDFSQGKDNTVGSYLKHFDLNPALAGHDIHIQFEGVERAMYVYLNGHFIGYAEDSFTPSEFDLTPYIQAKDNILAVEVFKHSTASWLEDQDMFRFSGIFRSVELLALPRTHLMDLDIKPTVVNDYHDGVFNAKLHFMGKTSGNVHVLIEDIDGKTLLNKKLPLKSTVEIENETFANVHLWDNHDPYLYQLIIEVHDQDGKLVELIPYQFGFRKIEITKDHVVLLNGKRLIINGVNRHEWDAKRGRSITLADMKQDIATFKHNNINAVRTCHYPNQIPWYYLCDQNGIYMMAENNLESHGTWQKLGQVEATSNVPGSIPEWREVVVDRARSNYETFKNHTAILFWSLGNESYAGSNIAAMNKLYKDHDSSRLTHYEGVFHAPEFKKEISDLESCMYLPPKEAEEYLQNPKKPLVECEYMHDMGTPDGGMGSYIKLIDKYPQYMGGFIWDFIDQALLVHDPVSGQDVLRYGGDFDDRHSDYEFSGDGLMFADRTPKPAMQEVRYYYGLHK

SEQ ID NO: 6 - protein, 316 aa, Lactobacillus amylovorus
MAYTNNLHVVYGEASLGVNGQDFAYLFSYERGGLESLKIKDKEWLYRTPTPTFWRATTDNDRGSGFNQKAAQWLGADMFTKCVGIHVQVDDHRFDELPVAPINNQFSNQEFAHEVKVAFDYETLTTPATKVKIIYNINDFGHMTITMHYFGKKGLPPLPVIGMRFIMPTKAKSFDYTGLSGETYPDRMAGAERGTFHIDGLPVTKYLVPQENGMHMQTNELVITRNSTQNNADKDGDFSLKITQTKQPFNFSLLPYTAEELENATHIEELPLARRSVLVIAGAVRGVGGIDSWGSDVEEQYHIDPEQDHEFSFTLN

SEQ ID NO: 7 - protein, 1052 aa, Bifidobacterium bifidum
MNTTDDQRKNGDPIVSPSIPTTAWLADPRVYAVHRLDAHSDHACWSRSPVDGESTDLRQSLDGEWRVRVETAPTGRFPDGTSDGPDWISDVSPLFAAPGFDDSSFSRVQVPSHLETAGLLAPQYVNVQYPWDGHEDPKAPAIPEHGHVAVYRREFDADGEVAQAVREGRPVTLTFQGAATAIYVWLNGSFIGYAEDSFTPSEFDVTDAIKVDGNVLAVACYEYSSASWLEDQDFWRLHGLFRSVELNARPAAHVADLHADADWDLATSRGSLSLDVLIDGAANAATADFALRDKNGTIVWRTATKADGTLHAEAEIDDAAPWSAERPDLYELSVTLLDADGKVLETARTRIGFRHVAIEDGILKLNGKRLVFRGVNRHEFDCRRGRAITEEDMLWDIRFMKRHNINAVRTSHYPNQSRWYELCDEYGIYLIDETNLETHGSWNSPGDIPVGTSVPGDDEAWLGACIDRLDSMILRDRNHPSVLVWSLGNESYAGEVLKAMSAHAHQLDPGRPVHYEGVNWNHAYDGISDFESRMYAKPAEIQDWLEHGDERGEASKPFVSCEYMHAMGNSCGGLSEFIDLERYERYSGGFIWDYIDQGLVQRLPDGSERLSVGGEWGDRPTDYEFVGNGIVFADRTPSPKAQEVKQLYSPVKLAPDGHGVTIENRNLFAGTDGYVFAARLLEDGHEIWHADYRFDVAAGDTQHHDIAFPDIDADGDTREVTYEVDLLLAEATAWAPAGYELAFGQLTGTLNPEQDITETSHDDDGRATRTLSRWNAGIRRDDEEILLSRTQGGIVSWKRDDREMVIRRPELVTFRPLTDNDRGNHSGFDRAAWFAAGRYAIVTETKIHESDDGLVAEYQYELADPNHTPVSVTYHVNSDMRMQLTVEYPGNATDMASLPAFGIEWELPGEYDRLRYYGPGPEETYRDRKQGGKLGIWDATAKASMAPYLMVQETGSHEDVRWLEATDIQGHGLRVTQRGDRHFTASLLPWNTYTIEAARRHEDLPKPRHNYLRLLAAQMGVGGDDSWGAPVHTAYQLPAGRPLTLDVNLELI

SEQ ID NO: 8 - protein, 1052 aa, Bifidobacterium bifidum
MNTTDDQRKNGDPIVSPSIPTTAWLADPRVYAVHRLDAHSDHACWSRSPVDGESTDLRQSLDGEWRVRVETAPTGRFPDGTSDGPDWISDVSPLFAAPGFDDSSFSRVQVPSHLETAGLLAPQYVNVQYPWDGHEDPKAPAIPEHGHVAVYRREFDADGEVAQAVREGRPVTLTFQGAATAIYVWLNGSFIGYAEDSFTPSEFDVTDAIKVDGNVLAVACYEYSSASWLEDQDFWRLHGLFRSVELNARPAAHVADLHADADWDLATSRGSLSLDVLIDGAANAATADFALWDKNGTIVWHIVTKADGTLHAEAEIDDAAPWSAERPDLYELSVTLLDADGKVLETARTRIGFRHVAIEDGILKLNGKRLVFRGVNRHEFDCRRGRAITEEDMLWDIRFMKRHNINAVRTSHYPNQSRWYELCDEYGIYLIDETNLETHGSWNSPGDIPVGTSVPGDDEAWLGACIDRLDSMILRDRNHPSVLVWSLGNESYAGEVLKAMSAHAHRLDPGRPVHYEGVNWNHAYDGISDFESRMYAKPAEIQDWLEHGDERGEASKPFVSCEYMHAMGNSCGGLSEFIDLERYERYSGGFIWDYIDQGLVQRLPDGSERLSVGGEWGDRPTDYEFVGNGIVFADRTPSPKAQEVKQLYSPVKLAPDGHGVTIENRNLFAGTDGYVFAARLLEDGHEIWHADYRFDVAAGDTQHHDIAFPDIDADGDTREVTYEVDLLLAEATAWAPAGYELAFGQLTGTLNPEQDITETSHDDDGRATRTLSRWNAGIRRDDKEILLSRTQGGIVSWKRDDREMVIRRPELVTFRPLTDNDRGNHSGFDRAAWFAAGRYAIVTETKIHESDDGLVAEYQYELADPNHTPVSVTYHVNSDMRMQLTVEYPGNATDMASLPAFGIEWELPGEYDRLRYYGPGPEETYRDRKQGGKLGIWDATAKASMAPYLMVQETGSHEDVRWLEATDIQGHGLRVTQRGDRHFTASLLPWNTYMIEAARRHEDLPEPRHNYLRLLAAQMGVGGDDSWGAPVHTAYQLPAGRPLTLDVNLELI

SEQ ID NO: 9 - protein, 1055 aa, Bifidobacterium breve
MTNSMQGKAKTIMTNLQSAQQFSQAWLTDPRVFAVNRLAAHSSHKFYDHSPQCGEAMDLKQSLDGQWRVQMLDLADLADNELAEAAFAQPGYDAAGFSPIEVPSALETKGFLNHQYVNQQYPWSGHESPVAPDVPKHNHVALYRHEFSLEPKAAAVLEANKTAADDAAKRRVTLTFQGAATAIVVWLNGAFIGYAEDSFTPSEFDVTDVLRDGVNTLAVACFEFSSASWLEDQDFWRLHGIFRSVELEAQPLVHVNDLRVLADYDHTTGEGSLDVVALLRNAGTAAAVAATVLDAAGNTVWHSKLTAGADAETLTVKANVGKVNPWSAEEPTLYTLQVVATDAAGQVIEAALQRIGFRHFAIEDGLMKLNGKRIVFKGVDRHEFDARTGRTIAEADMIEDIHSFKRLNINAVRTSHYPNETRWYELCDEYGIYVLDETNLETHGSWTDPGDVFQPARAIPGSKDEWRAACVDRTASMVRRDYNHPSVVIWSLGNEAFGGDVFYSMRDFVHENDPFRPVHYEGTFNDPEFSAATDIMSRMYAKPDEIVKLYLGEDGKKPYISCEYSHSMGNSTGGLHLYTELERYPLYQGGFIWDYVDQALWQDCGNGTERLAYGGDFEDRPNDYEFSGDGVMFADRTPSPKAQEVKQLYANVKLVPDESGVTITNDNLFISTASSLFTARVLVDGAERWHANYRFDVPAGETVREPIAFPKVTDLVALSGSAEVTYEVDQRLAEATDWAPAGYELTFGQYVAAVSFDDGAADAVVAGDAEVAADGFNAGIHTDFGEVLLSKTQGGMVSFKRDGREMVIRRPNLTTFRALTDNDRGNGSGFERAQWMAAGRYARVTGTSVEETADGKGLKATYSYELADAKHTPVTVHYEVDAALRVHLTVEYPGEADAATLPAFGLEWILPKQYDRLRFYGLGPEETYADRLHGAKLGVFSRTAAEDCAPYLLPQETGNHEQVRWAEITDEYGHGMRVTAAGGTRFATSLLPYSSLMFEDALHQNELPKPRHTFLRLLAAQMGVGGDDTWGAPVHDEFQVPADQPLKLDVTLELI

SEQ ID NO: 10 - protein, 689 aa, Bifidobacterium catenulatum
MTQRRSYRWPQPLAGQQARIWYGGDYNPDQWPEEVWDDDVRLMKKAGVNLVSVGIFSWAKIETSEGVYDFDWLDRIIDKLGEAGIAVDLASATASPPMWLTQAHPEVLWKDYRGDVCQPGARQHWRPTSPVFREYALKLCRAMAEHYKGNPYVVAWHVSNEYGCHNRFDYSEDAERAFRKWCEERYGTIDAVNDAWGTAFWAQRMNDFTEIVPPRFIGDGNFMNPGKLLDFKRFSSDALKAFYVAERDALAEITPDLPLTTNFMVSAAGSVLDYDDWGREVDFVSNDHYFIPGEAHLDELAFSASLVDGIARKDPWFLMEHSTSAVNWRPVNYRKEPGQLVRDSLAHVAMGADAVCYFQWRQSKAGAEKFHSAMVPHTGEDSAVFRDVCELGADLNTLADNGLLGTKLAKSKVAVVFDYESEWATEHTATPTQKVHHVDEPLQWFRALADHGVTADVVPVSSNWDEYEVVVLPSVYILSEETTRRVRDYVVNGGRLIVTYYTGLSDEKDHVWLGGYPGSIRDVVGVRVEEFMPMGDDFPGVPDCLGLSNGAVAHDIADVIGSVDGTATVLETFRDDPWTGMDGAPAIVANTFGEGRSVYVGARLGRDGIAKSLPEIFESLGMAETGENDSRVLRVEREGSDGSRFVFSFNRTHEAVQIPFEGKIVVSSFAEVSGENVSIKPNGVIVTKQ

SEQ ID NO: 11 - protein, 1023 aa, Bifidobacterium catenulatum
MANSNRVEHASETWLTDATVFEVNRTPAHSNHKCFTHDPQSGEHSDLTQSLDGEWRVEIVQASDIDFNEEPFVAENFDDSSFCRAQVPGHLQMAGLLKNKYVNIQYPWDGHENPLEPNVPENNHVALYRRKFVVSKRLADTKESEGSVSIVFHGMATAIYVWVNGLFAGYGEDGFTPNEFDITDLLHDGENVVAVACYEYSSASWLEDQDFWRLHGLFRSVELTAQPHVHVENMQLEADWDAESGTASLDAALSVRNASDAATISATLKDSEGNVVWEASTNADANTTFASGSLQGLEPWSAESPSLYELEVNVIDQAGNIVEAAVQKVGFRRFRIENGIMTLNGKRIVFKGADRHEFDAKRGRSITEQDMIDDVIFCKRHNINAIRTSHYPNQERWYDLCDEYGIYLIDETNLETHGSWCLPGDVVTAETAVPGSKAHWEGACVDRVNSMVRRDYNHPSVVIWSLGNESYTGDVFRAMYKHVHDIDPNRPVHYEGVTKNRDYDDVTDIETRMYEHADVVEEYLKNDPQKPYISCEYMHAMGNSVGNLDEYTALERYPHYQGGFIWDFIDQAIYATQPDGSTRLCYGGDFGDRPSDYEFSGNGLVFADRTPTPKAQEVKQLYSNVHIDVTDRSVSIKNDNLFISTGGYQFVLRILADGEPVWQSERRFDVPADSACTFDVEWPVDLYRANADELVLEVSQRLAEATDWAPAGYELAFGQTIVAGTKAAEDAALPADGIVTVGRWNAGVQGSGREILLSRTQGGLVSYTFDGHEFVLRRPAITTFRALTDNDRGAGHGFERAQWMVAGRYARCVDNVIEQVDEDTLKAVYTYELATPQCTKVTVGYTADTTGRLNLHVEYPGESGELPTIPAFGIEWTLPVQYSNLRFFGAGPEETYQDRKHAKLGVWSTDAFKDHAPYLMPQETGNHEEVRWAEITDENGHGLRVSRANGAAPFAVSLQPYSSFMIEEAQHQDELPAPKHMFLRVLAAQMGVGGDDSWMSPVHSQYHITADQPISLDVNLELI

SEQ ID NO: 12 - protein, 1008 aa, Lactobacillus delbrueckii subsp. bulgaricus
MSNKLVKEKRVDQADLAWLTDPEVYEVNTIPPHSDHESFQSQEELEEGKSSLVQSLDGDWLIDYAENGQGPVNFYAEDFDDSNFKSVKVPGNLELQGFGQPQYVNVQYPWDGSEEIFPPQIPSKNPLASYVRYFDLDEAFWDKEVSLKFDGAATAIYVWLNGHFVGYGEDSFTPSEFMVTKFLKKENNRLAVALYKYSSASWLEDQDFWRMSGLFRSVTLQAKPRLHLEDLKLTASLTDNYQKGKLEVEANIAYRLPNASFKLEVRDSEGDLVAEKLGPIRSEQLEFTLADLPVAAWSAEKPNLYQVRLYLYQAGSLLEVSRQEVGFRNFELKDGIMYLNGQRIVFKGANRHEFDSKLGRAITEEDMIWDIKTMKRSNINAVRCSHYPNQSLFYRLCDKYGLYVIDEANLESHGTWEKVGGHEDPSFNVPGDDQHWLGASLSRVKNMMARDKNHASILIWSLGNESYAGTVFAQMADYVRKADPTRVQHYEGVTHNRKFDDATQIESRMYAPAKVIEEYLTNKPAKPFISVEYAHAMGNSVGDLAAYTALEKYPHYQGGFIWDWIDQGLEKDGHLLYGGDFDDRPTDYEFCGNGLVFADRTESPKLANVKALYANLKLEVKDGQLFLKNDNLFTNSSSYYFLTSLLVDGKLTYQSRPLTFGLEPGESGTFALPWPEVADEKGEVVYRVTAHLKEDLPWADEGFTVAEAEEVAQKLPEFKPEGRPDLVDSDYNLGLKGNNFQILFSKVKGWPVSLKYAGREYLKRLPEFTFWRALTDNDRGAGYGYDLARWENAGKYARLKDISCEVKEDSVLVKTAFTLPVALKGDLTVTYEVDGRGKIAVTADFPGAEEAGLLPAFGLNLALPKELTDYRYYGLGPNESYPDRLEGNYLGIYQGAVKKNFSPYLRPQETGNRSKVRWYQLFDEKGGLEFTANGADLNLSALPYSAAQIEAADHAFDLTNNYTWVRALSAQMGVGGDDSWGQKVHPEFCLDAQKARQLRLVIQPLLLK

SEQ ID NO: 13 - protein, 1007 aa, Lactobacillus delbrueckii subsp. lactis
MSNKLVKEKRVDQADLAWLTDPEVYEVNTIPPHSDHESFQSQEELEEGKSSLVQSLDGNWLIDYAENGQGPINFYAEDFDDSNFKSVKVPGNLELQGFGQPQYVNIQYPWDGSEEIFPPQVPSKNPLASYVRYFDLDEALWDKEVSLKFAGAATAIYVWLNGHFVGYGEDSFTPSEFMVTKFLKKEGNRLAVALYKYSSASWLEDQDFWRLSGLFRSVTLEAKPLLHLEDLKLTASLTDNYQKGKLEVEANIAYRLPNASFKLEVRDSEGDLVAEKVGPIRSEKLGFSLADLPVAAWSAEKPNLYQVRLYLYQAGSLLEVSRQEVGFRNFELKDGIMYLNGQRIVFKGVNRHEFDSKLGRAITEADMIWDIKTMKQSNINAVRCSHYPNQSLFYRLCDKYGLYVIDEANLESHGTWEKVGHEDPSFNVPGDDQHWLGASLSRVKNMMARDKNHASILIWSLGNESYAGTVFAQMADYVRKADPTRVQHYEGVTHNRKFDDATQIESRMYAPAKEIEEYLTKKPAKPFISVEYAHAMGNSVGDLAAYTALEKYPHYQGGFIWDWIDQGLEKDGHLLYGGDFDDRPTDYEFCGDGLVFADRTTSPKLANVKALYSNLKLEVKDGQLFIKNDNLFTNSSAYYFLASLLVDGKLTYQSQPLTFGLEPGESGTFVLPWPEVEDEKGEIVYQVTAHLKEDLPWADEGFTVAEAEEAVTKLPEFYPAGRPELVDSDFNLGLKGNGFRILFSKAKGWPVSIKYAGREYLKRLPEFTFWRALTDNDRGAGYGYDLAKWENAGKYARLQDISYEIKENSALVKTTFTLPVALKGDLTITYEVDSLGKIAVTANFPGAVENGLLPAFGLNFALPKELSDYRYYGLGPNESYADRLEGSYLGIYQGAVEKNFTPYLRPQEAGNRSKVRYYQLFDEEGGLEFTANGADLNLSALPYSAAQIEAADHAFELTNNYTWVRALAAQMGVGGDDSWGQKVHPEFCLDAQEARQLKLVIQPLLLK

SEQ ID NO: 14 - protein, 1008 aa, Lactobacillus delbrueckii subsp. bulgaricus
MSNKLVKEKRVDQADLAWLTDPEVYEVNTIPPHFDHESFQSQEELEEGKSSLVQSLDGDWLIDYAENGQGPVNFYAEDFDDSNFKSVKVPGNLELQGFGQPQYVNVQYPWDGSEEIFPPQIPSKNPLASYVRYFDLDEAFWDKEVSLKFDGAATAIYVWLNGHFVGYGEDSFTPSEFMVTKFLKKENNRLAVALYKYSSASWLEDQDFWRMSGLFRSVTLQAKPRLHLEDLKLTASLTDNYQKGKLEVEANIAYRLPNASFKLEVRDSEGDLVAEKLGPIRSEQLEFTLADLPVAAWSAEKPNLYQVRLYLYQAGSLLEVSRQEVGFRNFELKDGIMYLNGQRIVFKGANRHEFDSKLGRAITEEDMIWDIKTMKRSNINAVRCSHYPNQSLFYRLCDKYGLYVIDEANLESHGTWEKVGGHEDPSFNVPGDDQHWLGASLSRVKNMMARDKNHASILIWSLGNESYAGTVFAQMADYVRKADPTRVQHYEGVTHNRKFDDATQIESRMYAPAKVIEEYLTNKPAKPFISVEYAHAMGNSVGDLAAYTALEKYPHYQGGFIWDWIDQGLEKDGHLLYGGDFDDRPTDYEFCGNGLVFADRTESPKLANVKALYANLKLEVKDGQLFLKNDNLFTNSSSYYFLTSLLVDGKLTYQSRPLTFGLEPGESGTFALPWPEVADEKGEVVYRVTAHLKEDLPWADEGFTVAEAEEVAQKLPEFKPEGRPDLVDSDYNLGLKGNNFQILFSKVKGWPVSLKYAGREYLKRLPEFTFWRALTDNDRGAGYGYDLARWENAGKYARLKDISCEVKEDSVLVKTAFTLPVALKGDLTVTYEVDGRGKIAVTADFPGAEEAGLLPAFGLNLALPKELTDYRYYGLGPNESYPDRLEGNYLGIYQGAVKKNFSPYLRPQETGNRSKVRWYQLFDEKGGLEFTANGADLNLSALPYSAAQIEAADHAFELTNNYTWVRALSAQMGVGGDDSWGQKVHPEFCLDAQKARQLRLVIQPLLLK

SEQ ID NO: 15 - protein, 1008 aa, Lactobacillus delbrueckii subsp. bulgaricus
MSNKLVKEKRVDQADLAWLTDPEVYEVNTIPPHSDHESFQSQEELEEGKSSLVQSLDGDWLIDYAENGQGPVNFYAEDFDDSNFKSVKVPGNLELQGFGQPQYVNVQYPWDGSEEIFPPQIPSKNPLASYVRYFDLDEAFWDKEVSLKFDGAATAIYVWLNGHFVGYGEDSFTPSEFMVTKFLKKENNRLAVALYKYSSASWLEDQDFWRMSGLFRSVTLQAKPRLHLEDLKLTASLTDNYQKGKLEVEANIAYRLPNASFKLEVRDSEGDLVAEKLGPIRSEQLEFTLADLPVAAWSAEKPNLYQVRLYLYQAGSLLEVSRQEVGFRNFELKDGIMYLNGQRIVFKGANRHEFDSKLGRAITEEDMIWDIKTMKRSNINAVRCSHYPNQSLFYRLCDKYGLYVIDEANLESHGTWEKVGGHEDPSFNVPGDDQHWLGASLSRVKNMMARDKNHASILIWSLGNESYAGTVFAQMADYVRKADPTRVQHYEGVTHNRKFDDATQIESRMYAPAKVIEEYLTNKPAKPFISVEYAHAMGNSVGDLAAYTALEKYPHYQGGFIWDWIDQGLEKDGHLLYGGDFDDRPTDYEFCGNGLVFADRTESPKLANVKALYANLKLEVKDGQLFLKNDNLFTNSSSYYFLTSLLVDGKLTYQSRPLTFGLEPGESGTFALPWPEVADEKGEVVYRVTAHLKEDLPWADEGFTVAEAEEVAQKLPEFKPEGRPDLVDSDYNLGLKGNNFQILFSKVKGWPVSLKYAGREYLKRLPEFTFWRALTDNDRGAGYGYDLARWENAGKYARLKDISCEVKEDSVLVKTAFTLPVALKGDLTVTYEVDGRGKIAVTADFPGAEEAGLLPAFGLNLALPKELTDYRYYGLGPNESYPDRLEGNYLGIYQGAVKKNFSPYLRPQETGNRSKVRWYQLFDEKGGLEFTANGADLNLSALPYSAAQIEAADHAFELTNNYTWVRALSAQMGVGGDDSWGQKVHPEFCLDAQKARQLRLVIQPLLLK

SEQ ID NO: 16 - protein, 1008 aa, Lactobacillus delbrueckii subsp. lactis
MSNKLVKEKRVDQADLAWLTDPEVYEVNTIPPHSDHESFQSQEELEEGKSSLVQSLDGDWLIDYAENGQGPVNFYAEDFDDSNFKSVKVPGNLELQGFGQPQYVNIQYPWDGSEEIFPPQVPSKNPLASYVRYFDLDEAFWDKEVSLKFAGAATAIYVWLNGHFVGYGEDSFTPSEFMVTKFLKKENNRLAVALYKYSSASWLEDQDFWRLSGLFRSVTLQAKPLLHLEDLKLTASLTDNYQKGKLEVEANIAYRLPNASFKLEVRDSEGDLVAEKLGPIRSEQLEFTLADLPVAAWSAEKPNLYQVRLYLYQAGSLLEVSRQEVGFRNFELKDGIMYLNGQRIVFKGVNRHEFDSKLGRAITEEDMIWDIKTMKRSNINAVRCSHYPNQSLFYRLCDKYGLYVIDEANLESHGTWEKVGHEDPSFNVPGDDQHWLGASLSRVKNMMARDKNHASILIWSLGNESYAGTVFAQMADYVRKADPTRVQHYEGVTHNRKFDDATQIESRMYAPAKEIEEYLTKKPAKPFISVEYAHAMGNSVGDLAAYTALEKYPHYQGGFIWDWIDQGLEKDGHLLYGGGDFDDRPTDYEFCGNGLVFADRTTSPKLANVKALYSNLKLEVKDGQLFLKNDNLFTNSSAYYFLTSLLVDGKLTYQSQPLTFGLEPGESGTFVLPWPEVEDEKGEIVYQVTAHLKEDLPWADEGFTVAEAEEAVTKLPEFYPAGRPELVDSDFNLGLKGNGFRILFSKAKGWPVSIKYAGREYLKRLPEFTFWRALTDNDRGAGYGYDLAKWENAGKYARLQDISYEIKENSVLVKTAFTLPVALKGDLTITYEVDSLGKIAVTANFPGAVENGLLPAFGLNFALPKELSDYRYYGLGPNESYADRLEGSYLGIYQGAVEKNFTPYLRPQEAGNRSKVRYYQLFDEESGLEFTANGADLNLSALPYSAAQIEAADHAFELSNNYTWVRALAAQMGVGGDDSWGQKVHPEFCLDAQEARQLKLVIQPLLLK

SEQ ID NO: 17 - protein, 1008 aa, Lactobacillus delbrueckii subsp. bulgaricus
MSNKLVKEKRVDQADLAWLTDPEVYEVNTIPPHSDHESFQSQEELEEGKSSLVQSLDGDWLIDYAENGQGPVNFYAEDFDDSNFKSVKVPGNLELQGFGQPQYVNVQYPWDGSEEIFPPQIPSKNPLASYVRYFDLDEAFWDKEVSLKFDGAATAIYVWLNGHFVGYGEDSFTPSEFMVTKFLKKENNRLAVALYKYSSASWLEDQDFWRMSGLFRSVTLQAKPRLHLEDLKLTASLTDNYQKGKLEVEANIAYRLPNASFKLEVRDSEGDLVAEKLGPIRSEQLEFTLADLPVAAWSAEKPNLYQVRLYLYQAGSLLEVSRQEVGFRNFELKDGIMYLNGQRIVFKGVNRHEFDSKLGRAITEEDMIWDIKTIKRSNINAVRCSHYPNQSLFYRLCDKYGLYVIDEANLESHGTWEKVGGHEDPSFNVPGDDQHWLGASLSRVKNMMARDKNHASILIWSLGNESYAGTVFAQMADYVRKADPTRVQHYEGVTHNRKFDDATQIESRMYAPAKVIEEYLTNKPAKPFISVEYAHAMGNSVGDLAAYTALEKYPHYQGGFIWDWIDQGLEKDGHLLYGGDFDDRPTDYEFCGNGLVFADRTESPKLANVKALYANLKLEVKDGQLFLKNDNLFTNSSSYYFLTSLLVDGKLTYQSRPLTFGLEPGESGTFALPWPEVADEKGEVVYRVTAHLKEDLPWADEGFTVAEAEEVAQKLPEFKPEGRPDLVDSDYNLGLKGNNFQILFSKVKGWPVSLKYAGREYLKRLPEFTFWRALTDNDRGAGYGYDLARWENAGKYARLKDISCEVKEDSVLVKTAFTLPVALKGDLTVTYEVDGRGKIAVTADFPGAEEAGLLPAFGLNLALPKELTDYRYYGLGPNESYPDRLEGNYLGIYQGAVKKNFSPYLRPQETGNRSKVRWYQLFDEKGGLEFTANGADLNLSALPYSAAQIEAADHAFDLTNNYTWVRALSAQMGVGGDDSWGQKVHPEFCLDAQKARQLRLVIQPLLLK

SEQ ID NO: 18 - protein, 1008 aa, Lactobacillus delbrueckii subsp. bulgaricus
MSNKLVKEKRVDQADLAWLTDPEVYEVNTIPPHSDHESFQSQEELEEGKSSLVQSLDGDWLIDYAENGQGPVNFYAEDFDDSNFKSVKVPGNLELQGFGQPQYVNVQYPWDGSEEIFPPQIPSKNPLASYVRYFDLDEAFWDKEVSLKFDGAATAIYVWLNGHFVGYGEDSFTPSEFMVTKFLKKENNRLAVALYKYSSASWLEDQDFWRMSGLFRSVTLQAKPRLHLEDLKLTASLTDNYQKGKLEVEANIAYRLPNASFKLEVRDSEGDLVAEKLGPIGSEQLEFTLADLPVAAWSAEKPNLYQVRLYLYQAGSLLEVSRQEVGFRNFELKDGIMYLNGQRIVFKGVNRHEFDSKLGRAITEEDMIWDIKTIKRSNINAVRCSHYPNQSLFYRLCDKYGLYVIDEANLESHGTWEKVGGHEDPSFNVPGDDQHWLGASLSRVKNMMARDKNHASILIWSLGNESYAGTVFAQMADYVRKADPTRVQHYEGVTHNRKFDDATQIESRMYAPAKVIEEYLTNKPAKPFISVEYAHAMGNSVGDLAAYTALEKYPHYQGGFIWDWIDQGLEKDGHLLYGGDFDDRPTDYEFCGNGLVFADRTESPKLANVKALYANLKLEVKDGQLFLKNDNLFTNSSSYYFLTSLLVDGKLTYQSRPLTFGLEPGESGTFALPWPEVADEKGEVVYRVTAHLKEDLPWADEGFTVAEAEEVAQKLPEFKPEGRPDLVDSDYNLGLKGNNFQILFSKVKGWPVSLKYAGREYLKRLPEFTFWRALTDNDRGAGYGYDLARWENAGKYARLKDISCEVKEDSVLVKTAFTLPVALKGDLTVTYEVDGRGKIAVTADFPGAEEAGLLPAFGLNLALPKELTDYRYYGLGPNESYPDRLEGNYLGIYQGAVKKNFSPYLRPQETGNRSKVRWYQLFDEKGGLEFTANGADLNLSALPYSAAQIEAADHAFELTNNYTWVRALSAQMGVGGDDSWGQKVHPEFCLDAQKARQLRLVIQPLLLK

SEQ ID NO: 19 - protein, 1007 aa, Lactobacillus delbrueckii subsp. lactis
MSNKLVKEKRVDQADLAWLTDPEVYEVNTIPPHSDHESFQSQEELEEGKSSLVQSLDGNWLIDYAENGQGPINFYAEDFDDSNFKSVKVPGNLELQGFGQPQYVNIQYPWDGSEEIFPPQVPSKNPLASYVRYFDLDEALWDKEVSLKFAGAATAIYVWLNGHFVGYGEDSFTPSEFMVTKFLKKEGNRLAVALYKYSSASWLEDQDFWRLSGLFRSVTLEAKPLLHLEDLKLTASLTDNYQKGKLEVEANIAYRLPNASFKLEVRDSEGDLVAEKVGPIRSEKLDFSLADLPVAAWSAEKPNLYQVRLYLYQAGSLLEVSRQEVGFRNFELKDGIMYLNGQRIVFKGVNRHEFDSKLGRAITEADMIWDIKTMKQSNINAVRCSHYPNQSLFYRLCDKYGLYVIDEANLESHGTWEKVGHEDPSFNVPGDDQHWLGASLSRVKNMMARDKNHASILIWSLGNESYAGTVFAQMADYVRKADPTRVQHYEGVTHNRKFDDATQIESRMYAPAKEIEEYLTKKPAKPFISVEYAHAMGNSVGDLAAYTALEKYPHYQGGFIWDWIDQGLEKDGHLLYGGDFDDRPTDYEFCGDGLVFADRTTSPKLANVKALYSNLKLEVKDGQLFIKNDNLFTNSSAYYFLTSLLVDGKLTYQSQPLTFGLEPGESGTFALPWPEVEDEKGEIVYQVTAHLKEDLPWADEGFTVAEAEEAVTKLPEFYPAGRPELVDSDFNLGLKGNGFRILFSKAKGWPVSIKYAGREYLKRLPEFTFWRALTDNDRGAGYGYDLAKWENAGKYARLQDISYEIKENSALVKTAFTLPVALKGDLTITYEVDSLGKIAVTANFPGAVENGLLPAFGLNFALPKELSDYRYYGLGPNESYADRLEGSYLGIYQGMVEKNFTPYLRPQEAGNRSKVRYYQLFDEEGGLEFTANGADLNLSALPYSAAQIEAADHAFELTNNYTWVRALAAQMGVGGDDSWGQKVHPEFCLDAQEARQLKLVIQPLLLK

SEQ ID NO: 20 - protein, 628 aa, Lactobacillus helvaticus
MQANINWLDNPEVFRVNQLPAHSDHPFFRDYREWQKQHSSYQQSLNGKWKFHFSANPMDRPQDFYQRDFDSSNFDSIPVPSEIELSNYTQNQYINVLFPWEGKIFRRPAYALDPNDHEEGSFSKGADNTVGSYLKRFDLSSALIGKDVHIKFEGVEQAMYVWLNGHFVGYAEDSFTPSEFDLTPYIQDKDNLLAVEVFKHSTASWLEDQDMFRFSGIFRSVELLGIPATHLMDMDLKPRVADNYQDGIFNLKLHFIGKKAGSFHLLVKDIKGHTLLEKNEDIKENVQINNEKFENVHLWNNHDPYLYQLLIEVYDEQQNLLELIPFQFGFRRIEISPEKVVLLNGKRLIINGVNRHEWDAKRGRSITMSDMTTDINTFKENNINAVRTCHYPNQIPWYYLCDQNGIYVMAENNLESHGTWQKMGEIEPSDNVPGSIPQWKEAVIDRARNNYETFKNHTSILFWSLGNESYAGDNIIAMNEFYKSHDDTRLVHYEGVVHRPELKDKISDVESCMYLPPKKVEEYLQNDPPKPFMECEYMHDMGNSDGGMGSYIKLLDKYPQYFGGFIWDFIDQALLVHDEISGHDVLRYGGDFDDRHSDYEFSGDGLMFADRTPKPAMQEVRYYYGLHK

SEQ ID NO: 21 - protein, 318 aa, Lactobacillus helvaticus
MDYTNNQLHIIYGDATFGVNGKDFQYIFSYERGGLESLKVHGKEWLYRVPTPTFWRATTDNDRGSGFNLKAAQWLGADMFTKCTDIHLKVDRHDFAELPIAPFNNKFSNHEYAKSAEISFTYQTLTTPATNAKIIYNIDDVGHIKVTMRYYGKKGLPPLPVIGIRLIMPTAATGFDYEGLSGETYPDRMAGAKEGKFHIDGLPVTEYLVPQENGMHMQTKKLTINRETTQNNVDRTNEKFSLSIQQAEKPFNFSCLPYTAEELENATHIEELPLVRRTVLVIAGAVRGVGGIDSWGTDVESAYHINPELDHEFSFILN

SEQ ID NO: 22 - protein, 1023 aa, Bifidobacterium longum
MTDVTHVDRASQAWLTDPTVFEVNRTPAHSSHKWYARDPQSGQWSDLKQSLDGEWRVEVVQAADINLEEEPATAESFDDSSFERIQVPGHLQTAGLMNHKYVNVQYPWDGHENPLEPNIPENNHVALYRRKFTVSAPVANAKQAGGSVSIVFHGMATAIYVWVNGAFVGYGEDGFTPNEFDITELLHDGENVVAVACYEYSSASWLEDQDFWRLHGLFRSVELAARPHVHIENTQIEADWDPEAGTASLDAALTVLNAADAATVRATLKDADGNTVWQTTGDAEAQTAISSGPLQGIAPWSAESPTLYELDVDVIDQAGDVIECTSQKVGFRRFRIEDGILTINGKRIVFKGADRHEFDAEQGRAITEQDMIDDVVFCKRHNINSIRTSHYPNQERWYELCDEYGIYLIDEANLEAHGSWSLPGDVLTEDTIVPGSKREWEGACVDRVNSMMRRDYNHPSVLIWSLGNESYVGDVFRAMYKHVHDIDPNRPVHYEGVTHNRDYDDVTDIETRMYSHADEIEKYLKDDPKKPYLSCEYMHAMGNSVGNMDEYTALERYPKYQGGFIWDFIDQAIYATQPDGTRSLRYGGDFGDRPSDYEFSGDGLLFANRKPSPKAQEVKQLYSNVHIDVTKDSVSVKNDNLFTATGDYVFVLSVLADGKPVWQSTRRFDVPAGETRTFDVAWPVAAYRADARELVLQVSQRLAKATDWAESGYELAFGQTVVPADATATPDTKPADGTITVGRWNAGVRGAGREVLLSRTQGGMVSYTFAGNEFVLRRPAITTFRPLTDNDRGAGHGFERVQWLGAGRYARCVDNVLEQIDDSTLKGTYTYELATAQRTKVTVSYTAHTDGRVNLHVEYPGEQGDLPTIPAFGIEWTLPVQYTNLRFFGTGPAETYLDRKHAKLGVWSTNAFADHAPYLMPQETGNHEDVRWAEITDDHGHGMRVSRADGAAPFAVSLLPYSSFMLEEAQHQDELPKPKHMFLRVLAAQMGVGGDDSWMSPVHPQYHIPADKPISLDVDLELI

SEQ ID NO: 23 - protein, 628 aa, Lactobacillus reuteri
MDADIKWLDEPETFRVNQLPAHSDHYYYGNYDEWRHNNSRFAQNLDGQWQFNFAENLRERENDFYKMDYDSSSFGTIEVPSEIELNNYAQNNYINTLIPWEGKIYRRPAYTLSPDDAQEGSFSDGDDNTIGEYLKHFDLDPSLRGKQVRIRFDGVERAMYVWLNGHFIGYAEDSFTPSEFDLTPYIQDEGNVLAVEVFKHSTASWIEDQDMFRFSGIFRSVNLLAQPLVHVEDLNIRPIVTDNYQDGIFNVELQLHGEKTGNVNVRVIDNDGNTLVNETHPVDSTVKVQDQFLENVHLWDNHDPYLYQLLIEIRDDEGNLVELVPYRFGFRRIEINKDHVVLLNGQRLIINGVNRHEWDARRGRAITMDDMTSDIHTFKENNINAVRTCHYPDQIPWYYLCDDNGIYMMAENNLESHATWQKMGAIEPSYNVPGSVPQWRDVVVDRARTNYETFKNHPSILFWSLGNESYAGDNIVKMNEFYKKHDDSRLVHYEGVCHTPEYRDRISDVESWMYLPPKEVEEYLKNNPDKPFMECEYMHDMGNSDGGMGSYISLLDKYPQYFGGFIWDFIDQALLVKDPVSGQEVMRYGGDFDDRHSDYEFSGDGLMFADRTPKPAMQEVRYYYGLHK

SEQ ID NO: 24 - protein, 319 aa, Lactobacillus reuteri
MAYTNKLRVIYGDATLGLSGDGFHYIFSYERGGLESLKLNGKEWLYREPMPTFWRATTDNDRGSGFNIRSAQWLAADTFHKCVGIDLTVDNQHFAELPIAPITNEFSDPVSAESVKIKYTFATLTVPATQVTVIYEVNGQGEIKVTMHYYGHEDLPGLPVVGMRFIMPTVATGFDYQGLSGETYPDRMAGATEGTFHVDGLPVTKYLVPQENGMHMATHALTITRDSTQNNADHSREPFSLTVKQDAQPFAFSCLPYTAEELENATHIEELPLARRTVLVVAGAVRGVGGIDSWGADVEEQYHIPADRDVEFSFVLNAK

SEQ ID NO: 25 - protein, 1007 aa, Lactobacillus delbrueckii subsp. lactis
MSNKLVKEKRVDQADLAWLTDPEVYEVNTIPPHSDHESFQSQEELEEGKSSLVQSLDGNWLIDYAENGQGPINFYAEDFDDSNFKSVKVPGNLELQGFGQPQYVNIQYPWDGSEEIFPPQVPSKIPLASYVRYFDLDEALWDKEVSLKFAGAATAIYVWLNGHFVGYGEDSFTPSEFMVTKFLKKEGNRLAVALYKYSSASWLEDQDFWRLSGLFRSVTLEAKPLLHLEDLKLTASLTDNYQKGKLEVEANIAYRLPNASFKLEVRDSEGDLVAEKVGPIRSEKLDFSLADLPVAAWSAEKPNLYQVRLYLYQAGSLLEVSRQEVGFRNFELKDGIMYLNGQRIVFKGVNRHEFDSKLGRAITEADMIWDIKTMKQSNINAVRCSHYPNQSLFYRLCDKYGLYVIDEANLESHGTWEKVGHEDPSFNVPGDDQHWLGASLSRVKNMMARDKNHASILIWSLGNESYAGTVFAQMADYVRKADPTRVQHYEGVTHNRKFDDATQIESRMYAPAKEIEEYLTKKPAKPFISVEYAHAMGNSVGDLAAYTALEKYPHYQGGFIWDWIDQGLEKDGHLLYGGDFDDRPTDYEFCGDGLVFADRTTSPKLANVKALYSNLKLEVKDGQLFIKNDNLFTNSSAYYFLTSLLVDGKLTYQSQPLTFGLEPGESGTFALPWPEVEDEKGEIVYQVTAHLKEDLPWADEGFTVAEAEEAVTKLPEFYPAGRPELVDSDFNLGLKGNGFRILFSKAKGWPVSIKYAGREYLKRLPEFTFWRALTDNDRGAGYGYDLAKWENAGKYARLQDISYEIKENSALVKTTFTLPVALKGDLTITYEVDSLGKIAVTANFPGAVENGLLPAFGLNFALPKELSDYRYYGLGPNESYADRLEGSYLGIYQGMVEKNFTPYLRPQEAGNRSKVRYYQLFDEEGGLEFTANGADLNLSALPYSAAQIEAADHAFELTNNYTWVRALAAQMGVGGDDSWGQKVHPEFCLDAQEARQLKLVIQPLLLK

SEQ ID NO: 26 - protein, 628 aa, Lactobacillus helvaticus
MQANINWLDNPEVFRVNQLPAHSDHPFFRDYREWQKQHSSYQQSLNGKWKFHFSANPMDRPQDFYQRDFDSSNFDSIPVPSEIELSNYTQNQYINVLFPWEGKIFRRPAYALDPNDHEEGSFSKGADNTVGSYLKRFDLSSALIGKDVHIKFEGVEQAMYVWLNGHFVGYAEDSFTPSEFDLTPYIQEKDNLLAVEVFKHSTASWLEDQDMFRFSGIFRSVELLGIPATHLMDMDLKPRVADNYQDGIFNLKLHFIGKKAGSFHLLVKDIKGHTLLEKNEDIKENVQINNEKFENVHLWNNHDPYLYQLLIEVYDEQQNLLELIPFQFGFRRIEISPEKVVLLNGKRLIINGVNRHEWDAKRGRSITMSDMTTDINTFKENNINAVRTCHYPNQIPWYYLCDQNGIYVMAENNLESHGTWQKMGEIEPSDNVPGSIPQWKEAVIDRARNNYETFKNHTSILFWSLGNESYAGDNIIAMNEFYKSHDDTRLVHYEGVVHRPELKDKISDVESCMYLPPKKVEEYLQNDPPKPFMECEYMHDMGNSNGGMDSYIKLLDKYPQYFGGFIWDFIDQALLVHDEISGHDVLRYGGDFDDRHSDYEFSGDGLMFADRKPKPAMQEVRYYYGLHK

SEQ ID NO: 27 - protein, 318 aa, Lactobacillus helvaticus
MDYTNNQLHIIYGDATFGVNGKDFQYIFSYERGGLESLKVHGKEWLYRVPTPTFWRATTDNDRGSGFNLKAAQWLGADMFTKCTDIHLKVDRHDFAELPIAPFNNKFSNHEYAKSAEISFTYQTLTTPATNAKIIYNIDDGGHIKVTMRYYGKKGLPPLPVIGIRLIMPTAATGFDYEGLSGETYPDRMAGAKEGKFHIDGLPVTEYLVPQENGMHMQTKKLTINRETTQNNVDRTNEKFSLSIQQAEKPFNFSCLPYTAEELENATHIEELPLVRRTVLVIAGAVRGVGGIDSWGTDVESAYHINPDLDHEFSFILN

SEQ ID NO: 28 - protein, 626 aa, Lactobacillus crispatus
MKANIKWLDDPEVFRINQLPAHSDHPFYKDYREWQKHSSSFKQSLNGAWQFHFSKDPQSRPIDFYKLSFDSSSFDTIPVPSEIELNGYAQNQYTNILYPWESKIYRKPAYTLGRGIKDGDFSQGKDNTVGSYLKHFDLNPALAGHDIHIQFEGVERAMYVYLNGHFIGYAEDSFTPSEFDLTPYIQAKDNILAVEVFKHSTASWLEDQDMFRFSGIFRSVELLALPRTHLMDLDIKPTVVNDYHDGVFNAKLHFMGKTSGNVHVLIEDIDGKTLLNKKLPLKSTVEIENETFANVHLWDNHDPYLYQLIIEVHDQDGKLVELIPYQFGFRKIEITKDHVVLLNGKRLIINGVNRHEWDAKRGRSITLADMKQDIATFKHNNINAVRTCHYPNQIPWYYLCDQNGIYMMAENNLESHGTWQKLGQVEATSNVPGSIPEWREVVVDRARSNYETFKNHTAILFWSLGNESYAGSNIAAMNKLYKDHDSSRLTHYEGVFHAPEFKKEISDLESCMYLPPKEAEEYLQNPKKPLVECEYMHDMGNSDGGIGSYIKLIDKYPQYMGGFIWDFIDQALLVHDPVSGQDVLRYGGDFDDRHSDYEFSGDGLMFADRTPKPAMQEVRYYYGLHK

SEQ ID NO: 29 - protein, 316 aa, Lactobacillus crispatus
MAYTNNLHVVYGEASLGVNGQDFAYLFSYERGVLESLKIKDKEWLYRTPTPTFWRATTDNDRGSGFNQKAAQWLGADMFTKCVGIHVQVDDHQFDELPIAPINNQFSNQEFAHEVKVAFDYETLTTPATKVKIIYNINDAGHMTITMHYFGKKGLPPLPVIGMRFIMPTKAKSFDYTGLSGETYPDRMAGAERGTFHIDGLPVTKYLVPQENGMHMQTNELVITRNSTQNNADKDGDFSLKITQTKQPFNFSLLPYTAEELENATHIEELPLARRSVLVIAGAVRGVGGIDSWGSDVEEQYHIDPEQDHEFSFTLN

SEQ ID NO: 30 - protein, 1025 aa, Streptococcus thermophilus
MNMTKIQTYLNDPKIVSVNTVDAHSDHKYFESLEEFSEGEMKLRQSLNGKWKIHYAQNTNQVLKDFYKTEFDETDLNFINVPGHLELQGFGSPQYVNTQYPWDGKEFLRPPQVPQESNAVASYVKHFTLNDALKDKKVFISFQGVATSIFVWVNGNFVGYSEDSFTPSEFEISDYLVEGDNKLAVAVYRYSTASWLEDQDFWRLYGIFRDVYLYAIPKVHVQDLFVKGDYDYQTKAGQLDIDLKTVGDYEDKKIKYVLSDYEGIVTEGDASVNGDGELSVSLENLKIKPWSAESPKLYDLILHVLDDDQVVEVVPVKVGFRRFEIKDKLMLLNGKRIVFKGVNRHEFNARTGRCITEEDMLWDIKVMKQHNINAVRTSHYPNQTRWYELCDEYGLYVIDEANLETHGTWQKLGLCEPSWNIPASEPEWLPACLDRANNMFQRDKNHASVIIWSCGNESYAGKDIADMADYFRSVDNTRPVHYEGVAWCREFDYITDIESRMYAKPADIEEYLTTGKLVDLSSVSDKHFASGNLTNKPQKPYISCEYMHTMGNSGGGLQLYTDLEKYPEYQGGFIWDFIDQAIYKTLPNGSEFLSYGGDWHDRPSDYEFCGNGIVFADRTLTPKLQTVKHLYSNIKIAVDEKSVTIKNDNLFEDLSAYTFLARVYEDGRKVSESEYHFDVKPGEEATFPVNFVVEASNSEQIYEVACVLREATKWAPKGHEIVRGQYVVEKISTETPVKAPLNVVEGDFNIGIQGQNFSILLSRAQNTLVSAKYNGVEFIEKGPKLSFTRAYTDNDRGAGYPFEMAGWKVAGNYSKVTDTQIQIEDDSVKVTYVHELPGLSDVEVKVTYQVDYKGRIFVTANYDGKAGLPNFPEFGLEFAIGSQFTNLSYYGYGAEESYRDKLPGAYLGRYETSVEKTFAPYLMPQESGNHYGTREFTVSDDNHNGLKFTALNKAFEFSALRNSTEQIENARHQYELQESDATWIKVLAAQMGVGGDDSWGAPVHDEFLLSSADSYQLSFMIEPLN

SEQ ID NO: 31 - protein, 1008 aa, Lactobacillus delbrueckii subsp. indicus
MNNKLAQVKRVDQADLAWLTDPEIYEVNTIPPHSDHESFQSLEELEEGKSSLVQSLDGDWLIDYAENGEGPANFYEENFDDSSFKSVKVPGNLELQGFGQPQYVNVQYPWDGSDEIFPPMIPSKNPVASYVRYFDLEEAFWDKEVSLKFAGAATAIYVWLNGHFVGYGEDSFTPSEFMVTKFLKKEGNRLAVALYKYSSASWLEDQDFWRMSGLFRSVTLEAKPLLHLQDLKLTASLTNDYQKGSLQVEADIDYRLPNSSFKLELRDSAGELVAEKVGPIRSEKLDFSLADLPVAAWSAEEPNLYQVRLSLYQQGSLLEVSRQEVGFRNFELKDGIMYLNGKRIVFKGVNRHEFDSKLGRAITEADMIWDIKTMKQSNINAVRCSHYPNQSIFYHLCDKYGLYVIDEANLESHGTWEKVGGHEDPSFNVPGDDQRWLGASLSRVKNMMARDKNHASILIWSLGNESYAGKVFAQMADYVRQADPTRVQHYEGVTHNRKFDDATQIESRMYAPAKEIEEYLTKKPAKPFVSCEYAHAMGNSVGDLAAYTALEKYPHYQGGFIWDWIDQGLEKEGHLLYGGDFDDRPSDYEFCGDGLVFADRTTSPKLANVKALYSNLKLELKDGQLFLKNDNLFTNSSAYYFLTSLLVDGKLTYQSQPLTFALEPGESGTFALPWPEVEDEKGEIVYQVTAHLKEDLPWADEGFTVAEAEEAVTKLPEFYPAGRPELVDSDYNLGIKGNGFRILFSKAKGWPVSIKYAGREYLKRLPEFTFWRALTDNDRGAGYGYDLAKWENAGKYARLQDISYEIKENSVLVKTAFTLPVALKGDLTITYEVDSLGKIAVTANFPGAVENGLLPAFGLNFALPKELSDYRYYGLGPNESYADRLEGSYLGIYQGAVEKNFTPYLRPQEVGNRSKVRYYQLFDEEGGLEFTANGANLNLSALPYSAAQIEAADHAFELTNNYTWVRALAAQMGVGGDDSWGQKVHPEFCLDAQEARQLKLVIQPLFTE

SEQ ID NO: 32 - protein, 1049 aa, Bifidobacterium adolescentis
MADTAELAIVHATTASASWLTDPTVFAANRKPAHSSHRYVIGETSEPKQSLDGEWKVRIEQARNVDVESAPFAAVDFEDGDFGAIEVPGHLQMAGYLKNKYVNIQYPWDGHEDPQAPNIPENNHVAIYRRRFALDAQLARTLENDGTVSLTFHGAATAIYVWLDGTFVGYGEDGFTPSEFDVTEALRNGNGNAADSPEAEHTLTVACYEYSSASWLEDQDFWRLHGLFRTVELAAQPHTHVETVQLEADYTAADTAGTADTAELNAALTLRNPADAMTIESTLRDGDGNVVWESTQACNGEIALNSGKMTNIAPWSAESPTLYTLTVRVVGHDGAIIETVTQKIGFRTFRIENGIMTLNGKRIVFKGADRHEFDAKRGRAITREDMLSDVVFCKRHNINAIRTSHYPNQEYWYDLCDEYGLYLIDETNMETHGTWVANNVERPEDGIPGSRPEWEDACVDRINSMMRRDYNHPSVLIWSLGNESSAGEVFRAMYRHAHTIDPNRPVHYEGSVHMREFEDVTDIESRMYAHADEIERYLNDGSPAHTDGPKKPYISCEYMHAMGNSCGNMDEYTALERYPMYQGGFIWDFIDQAIETKLPDGTTRMCYGGDFGDRPSDYEFSGDGLLFADRTPSPKAQEVKQLYANVKIAVSVDEARITNDNLFVSTGDYRFVLRILADGKPVWSTTRRFDVAAGESASFEVDWPVDDYRSNAEELVLEVSQQLGNACDWAPAGYELAFGQCVVAGAKTTADAVDAAGAPADGTVTLGRWNAGVRGQGREALFSRTQGGMVSYTFGEREFVLRRPSITTFRPLTDNDRGAGHAFERAAWAVAGKYARCVDCAIANRGENAVEATYTYELAIPQRTKVTVRYVADTAGLVSLDVEYPGEKNGDLPTIPAFGIEWALPVEYANLRFYGAGPEETYADRRHAKLGVWSTTAGDDCAPYLLPQETGNHEDVRWAEITDDSGHGVRVKRGAGAKPFAMSLLPYSSTMLEEALHQDELPKPRHMFLRLLAAQMGVGGDDSWMSPVHEQYQLPADQPLSLNVQLKLF

SEQ ID NO: 33 - protein, 1023 aa, Bifidobacterium adolescentis
MANETRIEHASETWLADSTVFEVNRVPAHSDHKCYAHDSQTNEWSDLRQSLDGEWRVEVVQASDIEFNEEPFVRENFDDSAFERIQVPGHLQMAGLMNNKYVNIQYPWDGHENPAEPNIPENNHVALYRKTFTMANRLADTKNAGGTVSIVFHGMATAIYVWVNGMFVGYGEDGFTPNEFDITEMLHDGENVVAVACYEYSSASWLEDQDFWRLHGLFRSVELAAQPHVHIENMQIESDWDPESGSASLDAALTVRNAADAATISATLKDSDGNVVWETANCADPDTSISTGSLNGIRPWSAEDPVLYEFEVTVIDHAGNIAEVAVQKVGFRRFRIEDGIMTINGKRIVFKGADRHEFDPKRGRAITEQDMIDDVVFCKRHNLNAIRTSHYPNQERWYELCDEYGIYLIDETNLETHGSWCLPGDVLTEETAVPGSKAHWEGACVDRVNSMVRRDYNHPSVLIWSLGNESYTGDVFRAMYKRVHDIDPNRPVHYEGVTHNRDYNDVTDIETRMYAHADAIEEYLKNDPQKPYISCEYMHAMGNSCGNMDEYTALERYPKYQGGFIWDFIDQAIYATQPDGTTSLRYGGDFGDRPSDYEFSGNGLVFADRKPTPKAQEVKQLYSNVHIDVAEDSVTIKNDNLFTSTGEYTFVLRVLADGEPVWQSERRFDVPAGSTEKLDVDWPLDLYRDGASELVLEVSQRLAKATNWAVAGYELAFGQTVVAGSKKASAPVKPVDGIVTVGRWNVGVQGSGREVLLSRTQGGLVSYTFNNREFVLRRPAVTTFRALTDNDRGAGHGFERAQWLGAGRYARCIGNEIEQIDENTVKASYTYELATPQRTKVTVSYTADTTGRVNLHVEYPGEPGDLPTIPAFGIEWTLPVQYSNLRFFGAGPEETYQDRKHAKLGVWSTDAFKDHAPYLMPQETGNHEDVRWAEITDEKGHGLRISRAEGAEPFAMSLQPYSSFMLEEAQHQDELPAPKHMFLRVLAEQMGVGGDDSWMSPVHPQYHIPADQPISLDVDLDLI

SEQ ID NO: 34 - protein, 1305 aa, Bifidobacterium bifidum
MVEDATRSDSTTQMSSTPEVVYSSAVDSKQNRTSDFDANWKFMLSDSVQAQDPAFDDSAWQQVDLPHDYSITQKYSQSNEAESAYLPGGTGWYRKSFTIDRDLAGKRIAINFDGVYMNATVWFNGVKLGTHPYGYSPFSFDLTGNAKFGGENTIVVKVENRLPSSRWYSGSGIYRDVTLTVTDGVHVGNNGVAIKTPSLATQNGGNVTMNLTTKVANDTEAAANITLKQTVFPKGGKTDAAIGTVTTASKSIAAGASADVTSTITAASPKLWSIKNPNLYTVRTEVLNGDTVLDTYDTEYGFRWTGFDATSGFSLNGEKVKLKGVSMHHDQGSLGAVANRRAIERQVEILQKMGVNSIRTTHNPAAKALIDVCNEKGVLVVEEVFDMWNRSKNGNTEDYGKWFGQTIAGDNAVLGGDKDETWAKFDLTSTINRDRNAPSVIMWSLGNEMMEGISGSVSDFPATSAKLVAWTKAADSTRPMTYGDNKIKANWNESNTMGDNLTANGGVVGTNYSDGANYDKIRTTHPSWAIYGSETASAINSRGIYNRTTGGAQSSDKQLTSYDNSAVGWGAVASSAWYDVVQRDFVAGTYVWTGFDYLGEPTPWNGTGSGAVGSWPSPKNSYFGIVDTAGFPKDTYYFYQSQWNDDVHTLHILPAWNENVVAKGSGNKVPVVVYTDAAKVKLYFTPKGSTEKRLIGEKSFTKKTTAAGYTYQVYEGTDKDSTAHKNMYLTWNVPWAEGTISAEAYDENNRLIPEGSTEGNASVTTTGKAAKLKADADRKTITADGKDLSYIEVDVTDANGHIVPDAANRVTFDVKGAGKLVGVDNGSSPDHDSYQADNRKAFSGKVLAIVQSTKEAGEITVTAKADGLQSSTVKIATTAVPGTSTEKTVRSFYYSRNYYVKTGNKPILPSDVEVRYSDGTSDRQNVTWDAVSDDQIAKAGSFSVAGTVAGQKISVRVTMIDEIGALLNYSASTPVGTPAVLPGSRPAVLPDGTVTSANFAVHWTKPADTVYNTAGTVKVPGTATVFGKEFKVTATIRVQRSQVTIGSSVSGNALRLTQNIPADKQSDTLDAIKDGSTTVDANTGGGANPSAWTNWAYSKAGHNTAEITFEYATEQQLGQIVMYFFRDSNAVRFPDAGKTKIQISADGKNWTDLAATETIAAQESSDRVKPYTYDFAPVGATFVKVTVTNADTTTPSGVVCAGLTEIELKTATSKFVTNTSAALSSLTVNGTKVSDSVLAAGSYNTPAIIADVKAEGEGNASVTVLPAHDNVIRVITESEDHVTRKTFTINLGTEQEFPADSDERD

SEQ ID NO: 35 - protein, 1025 aa, Kluyveromyces lactis
MSCLIPENLRNPKKVHENRLPTRAYYYDQDIFESLNGPWAFALFDAPLDAPDAKNLDWETAKKWSTISVPSHWELQEDWKYGKPIYTNVQYPIPIDIPNPPTVNPTGVYARTFELDSKSIESFEHRLRFEGVDNCYELYVNGQYVGFNKGSRNGAEFDIQKYVSEGENLVVVKVFKWSDSTYIEDQDQWWLSGIYRDVSLLKLPKKAHIEDVRVTTTFVDSQYQDAELSVKVDVQGSSYDHINFTLYEPEDGSKVYDASSLLNEENGNTTFSTKEFISFSTKKNEETAFKINVKAPEHWTAENPTLYKYQLDLIGSDGSVIQSIKHHVGFRQVELKDGNITVNGKDILFRGVNRHDHHPRFGRAVPLDFVVRDLILMKKFNINAVRNSHYPNHPKVYDLFDKLGFWVIDEADLETHGVQEPFNRHTNLEAEYPDTKNKLYDVNAHYLSDNPEYEVAYLDRASQLVLRDVNHPSIIIWSLGNEACYGRNHKAMYKLIKQLDPTRLVHYEGDLNALSADIFSFMYPTFEIMERWRKNHTDENGKFEKPLILCEYGHAMGNGPGSLKEYQELFYKEKFYQGGFIWEWANHGIEFEDVSTADGKLHKAYAYGGDFKEEVHDGVFIMDGLCNSEHNPTPGLVEYKKVIEPVHIKIAHGSVTITNKHDFITTDHLLFIDKDTGKTIDVPSLKPEESVTIPSDTTYVVAVLKDDAGVLKAGHEIAWGQAELPLKVPDFVTETAEKAAKINDGKRYVSVESSGLHFILDKLLGKIESLKVKGKEISSKFEGSSITFWRPPTNNDEPRDFKNWKKYNIDLMKQNIHGVSVEKGSNGSLAVVTVNSRISPVVFYYGFETVQKYTIFANKINLNTSMKLTGEYQPPDFPRVGYEFWLGDSYESFEWLGRGPGESYPDKKESQRFGLYDSKDVEEFVYDYPQENGNHTDTHFLNIKFEGAGKLSIFQKEKPFNFKISDEYGVDEAAHACDVKRYGRHYLRLDHAIHGVGSEACGPAVLDQYRLKAQDFNFEFDLAFE

SEQ ID NO: 36 - DNA, 30 bp, Primer
  misc_feature (9)..(9): n is a deoxyuracil residue at 9th positions
attaaccangcgacgcaacttcgaatggcc

SEQ ID NO: 37 - DNA, 31 bp, Primer
  misc_feature (9)..(9): n is a deoxyuracil residue at 9th positions
atcttctcnttaccgccttaccacgagcacg

SEQ ID NO: 38 - DNA, 33 bp, Primer
  misc_feature (9)..(9): n is a deoxyuracil residue at 9th positions
agagaagantttcagcctgatacagattaaatc

SEQ ID NO: 39 - DNA, 33 bp, Primer
  misc_feature (9)..(9): n is a deoxyuracil residue at 9th positions
atggttaantcctcctgttagcccaaaaaacgg

SEQ ID NO: 40 - DNA, 22 bp, Primer
cggcgtcacactttgctatgcc

SEQ ID NO: 41 - DNA, 20 bp, Primer
ccgcgctactgccgccaggc